European Patent Application EP 4 703 721 A1, published March 4, 2026. Title: Methods for detecting cashew nuts. Applicant: NISSIN FOODS HOLDINGS. Application JP 000226976, filed April 27, 2023. The sequence listing filed with the application follows.

SEQUENCE LISTING (3 sequences)

SEQ ID NO: 1 - protein, 12 aa, cashew nuts
GSESEEESEDEK

SEQ ID NO: 2 - protein, 12 aa, cashew nuts
GQVQVVDNFGNR

SEQ ID NO: 3 - protein, 12 aa, cashew nuts
DVFQQQQQHQSR